European Patent Application EP 4 130 276 A1, published February 8, 2023. Title: Protein having peptidoglycan degrading activity, DNA encoding same, preparation and method for decomposing microorganisms. Applicant: SUMITOMO CHEMICAL COMPANY, LIMITED Kataoka Bio Laboratory Co., LTD. The sequence listing filed with the application follows.

SEQUENCE LISTING (26 sequences)

SEQ ID NO: 1 - DNA, 699 bp, Tumebacillus sp. NITE BP-02779
  CDS (1)..(696)
  mat_peptide (205)..(696)
atgaaaaaagcatctgcactgctgttgatgacagctgcaatgtccctcgtggcaacctccgcgatggcaaccccggctgtgaaggaagtcaaacaaaaagacggctccgttcgtctcgacgttgcagaacgtccgtccaacggcaccccggaagcacaacaaggcacgaaactcgtggttgacccgcaaggcgtgaccgcagcagcggcgtacaccaagccgtccacgatccgcgtcgggattcgtgcgaacaacaacaccgcgaacccgatcggttccgtatcggttgttccgtggtatgactacaacatcgacgtgctcccgaacgagtggatcggctcttggccggcacaatcgctcaacgcaggcgcgatcgcagtaaaaatgtacgcttggtatcatatccttcatccgaaatactccacctgtgacgttgataacacggtaaactcccaagtttacaaagcaggctcccgctatagcaacaccacgaccgctgttgataacatgtccggcatcggcatcctcaaaagcggcgtgatgttcgaaacccaataccgtgctggctcgtacgattcctcgatcccgggcacgaacattatgtcccaaaacggtacccactactacgcagaccaaggcaaaacttggtcttggatgacgaactactactacccgggttccgcacaattcacctactaa

SEQ ID NO: 2 - protein, 232 aa, Tumebacillus sp. NITE BP-02779
MKKASALLLMTAAMSLVATSAMATPAVKEVKQKDGSVRLDVAERPSNGTPEAQQGTKLVVDPQGVTAAAAYTKPSTIRVGIRANNNTANPIGSVSVVPWYDYNIDVLPNEWIGSWPAQSLNAGAIAVKMYAWYHILHPKYSTCDVDNTVNSQVYKAGSRYSNTTTAVDNMSGIGILKSGVMFETQYRAGSYDSSIPGTNIMSQNGTHYYADQGKTWSWMTNYYYPGSAQFTY

SEQ ID NO: 3 - DNA, 1566 bp, Tumebacillus sp. NITE BP-02779
  CDS (1)..(1563)
  mat_peptide (85)..(1563)
atgaaaaaaacttgggtttcggtccttgcgaccaccgcgctgacgctgtcggttggcagcgtatacgcgcaacctgcgcatgcagaacagtctaccaaacaatcggtcgccactgcacccgttctggaaagcgcattcacatccgctgcgaaggaatttggcgttccgaaggacctgctgatggcgatctcctatagcgagtcgcgctggcagatcgcgccagaggaagcccgcactagctcggagccggataaaaacaacggcaagggtctgatgcacctccaggacaactccttcaaaaaaggtctgagcgaagcagcaaaagcgctcggcgtttccaaaaaacagatggaagatgacatccaattgaatatccgcggcggtgcctacctgctgtcaaaagcacaaaaagacctcggcaagacgctcaccgccaacgcgaacgattggtacgaagcggtcgcttccttcgaaggagccaaggacaaggacctcggcgcactgttcgctgacgaagtgtaccgtgtgctgaaggaaggcacggcgctggcgatctctggcggcacgctgacgctcgacccgaacaaatcgatcgctccagccaaaggctcctacgcaggcttgatcccaggtggtacgaactacggactgaccccggactactccggcgcgatctggaacccggccagctcgtcgaactatgcggttgcctcccgccccacatcgaacgcgatcacctcggtcatcatccatgacaccgagggttcctactccggatcgatcaactggttcaaagacccggcggcgcaagtttccgcgcactacatcgtccgttcctccgacgggcaaatcacgcagttggtccaagacaaggacatcgcgtggcatgcgcgcaccttcaacaccaacggcatcggcatcgagcacgagggctatgcggcccaaaccggctggtacaccgatgcgatgtacactgcatcggcggcgctcacccgtgcagtctgtctcaaatacaacatcccgatggaccgcgaacacatcatggcacactctgaactctggggcaacgaccacaccgatccgggcgtgaactgggactggaacaaatacatgagcaaagtcaccggcgtcacgaaaaactacgatgccgtgctggtcgacaacacagacgcctcctccggcttctcgctgggcggcccgtcccagtattggcatccgaccgctggctacggcatccacaaccagatgacctacacgatgggcaatggcaccaacccgatctccaactacgcgacgtggagaccgacgatcacgacctcgggcaactaccaagtgaaagtcttcatcccgtccaacttcgccgcgaccaccaacgcgaagtacgagatccattacaacggcggcgtgatcaccaagacgatctcccaagccgcatactccaaccaatgggtgagcctcggcacctacagttttgcagccggcaccaccggctacgtcatgttgggtgacaacaccggcgacaaagcgtacgtcggcattgacggcatgcgtttcctcgctcaataa

SEQ ID NO: 4 - protein, 521 aa, Tumebacillus sp. NITE BP-02779
MKKTWVSVLATTALTLSVGSVYAQPAHAEQSTKQSVATAPVLESAFTSAAKEFGVPKDLLMAISYSESRWQIAPEEARTSSEPDKNNGKGLMHLQDNSFKKGLSEAAKALGVSKKQMEDDIQLNIRGGAYLLSKAQKDLGKTLTANANDWYEAVASFEGAKDKDLGALFADEVYRVLKEGTALAISGGTLTLDPNKSIAPAKGSYAGLIPGGTNYGLTPDYSGAIWNPASSSNYAVASRPTSNAITSVIIHDTEGSYSGSINWFKDPAAQVSAHYIVRSSDGQITQLVQDKDIAWHARTFNTNGIGIEHEGYAAQTGWYTDAMYTASAALTRAVCLKYNIPMDREHIMAHSELWGNDHTDPGVNWDWNKYMSKVTGVTKNYDAVLVDNTDASSGFSLGGPSQYWHPTAGYGIHNQMTYTMGNGTNPISNYATWRPTITTSGNYQVKVFIPSNFAATTNAKYEIHYNGGVITKTISQAAYSNQWVSLGTYSFAAGTTGYVMLGDNTGDKAYVGIDGMRFLAQ

SEQ ID NO: 5 - DNA, 20 bp, Artificial Sequence
  27F, primer for 16S rRNA cloning
agrgtttgatcmtggctcag

SEQ ID NO: 6 - DNA, 19 bp, Artificial Sequence
  1492R, primer for 16S rRNA cloning
ggytaccttgttacgactt

SEQ ID NO: 7 - DNA, 19 bp, Artificial Sequence
  339F, primer for 16S rRNA sequencing
ctcctacgggaggcagcag

SEQ ID NO: 8 - DNA, 18 bp, Artificial Sequence
  536R, primer for 16S rRNA sequencing
gtattaccgcggctgctg

SEQ ID NO: 9 - DNA, 20 bp, Artificial Sequence
  907F, primer for 16S rRNA sequencing
aaactyaaaggaattgacgg

SEQ ID NO: 10 - DNA, 1471 bp, Tumebacillus sp. NITE BP-02779
acgaacgctggcggcgtgcctaatacatgcaagtcgagcggagtgtmgagagcttgctctcwraggtcagcggcggacgggtgagtaacacgtgggtaacctgcctggcagactgggataacgcttggaaacgagtgctaataccggataatctcttggatcgcatggtctgagagtaaaaggagcttttgcttcactgcyagatggacccgcggcgcattagctagttggtgaggtaatggctcaccaaggcgacgatgcgtagccgacctgagagggtgaccggccacactgggactgagacacggcccagactcctacgggaggcagcagtagggaatcttccgcaatgggcgcaagcctgacggagcaacgccgcgtgagtgatgaaggccttcgggttgtaaaactctgtcttctgtgaagaaccatcctgtgcagagaaagctcaggacctgacggtaacagaggaggaagccccggctaactacgtgccagcagccgcggtaatacgtagggggcaagcgttgtccggaatcactgggcgtaaagcgcgcgcaggcggtctctcacgtccggggtgaaagcccagagctcaactctgggattgccttggatacggggagacttgaggatcggagaggcaaggggaattccacgtgtagcggtgaaatgcgtagagatgtggaggaacacctgtggcgaaggcgccttgctggccgatttctgacgctgaggcgcgaaagcgtggggagcaaacaggattagataccctggtagtccacgccgtaaacgatgagtgctaggtgttagggggcccaccccttagtgccgaagctaacgcattaagcactccgcctggggagtacggtcgcaagactgaaactcaaaggaattgacgggggcccgcacaagcagtggagcatgtggtttaattcgaagcaacgcgaagaaccttaccaagacttgacatcccgctgaccrctctagagatagagyttcccttcggggcagcggtgacaggtggtgcatggttgtcgtcagctcgtgtcgtgagatgttgggttaagtcccgcaacgagcgcaacccctatgttgtgttgctaccatttagttgagcacttacaacagactgccggtgacaaaccggaggaaggcggggatgacgtcaaatcatcatgccccttatgtcttgggctacacacgtgctacaatggacggtacaaagggttgcgaagccgcgaggtgaagccaatcccagaaagccgttcgtagttcggattgcaggctgcaactcgcctgcatgaagccggaattgctagtaatcgcggatcagcatgccgcggtgaattcgttcccgggccttgtacacaccgcccgtcacaccatgggagttggtaacacccgaagtcggtgaggtaactgcttgcagagccagccgcctaaggtgggatcgataactggggtgaag

SEQ ID NO: 11 - protein, 46 aa, Tumebacillus sp. NITE BP-02779
ANNNTANPIGSVSVVPWYDYNIDVLPNEWIGSWPAQSLNAGAIAVK

SEQ ID NO: 12 - protein, 11 aa, Tumebacillus sp. NITE BP-02779
MYAWYHILHPK

SEQ ID NO: 13 - protein, 16 aa, Tumebacillus sp. NITE BP-02779
YSTCDVDNTVNSQVYK

SEQ ID NO: 14 - protein, 18 aa, Tumebacillus sp. NITE BP-02779
YSNTTTAVDNMSGIGILK

SEQ ID NO: 15 - protein, 10 aa, Tumebacillus sp. NITE BP-02779
SGVMFETQYR

SEQ ID NO: 16 - protein, 27 aa, Tumebacillus sp. NITE BP-02779
AGSYDSSIPGTNIMSQNGTHYYADQGK

SEQ ID NO: 17 - protein, 18 aa, Tumebacillus sp. NITE BP-02779
TWSWMTNYYYPGSAQFTY

SEQ ID NO: 18 - protein, 10 aa, Tumebacillus sp. NITE BP-02779
AAYTKPSTIR

SEQ ID NO: 19 - DNA, 31 bp, Artificial Sequence
  F primer for ID2839 cloning
atatacatatggcgtacaccaagccgtccac

SEQ ID NO: 20 - DNA, 31 bp, Artificial Sequence
  R primer for ID2839 cloning
ccctcgagttagtaggtgaattgtgcggaac

SEQ ID NO: 21 - protein, 20 aa, Artificial Sequence
  His_Tb restriction site
MGSSHHHHHHSSGLVPRGSH

SEQ ID NO: 22 - DNA, 33 bp, Artificial Sequence
  F primer for ID1644 cloning
cgccatatggaacagtctaccaaacaatcggtc

SEQ ID NO: 23 - DNA, 27 bp, Artificial Sequence
  R primer for ID1644 cloning
ccctcgagttattgagcgaggaaacgc

SEQ ID NO: 24 - DNA, 35 bp, Artificial Sequence
  F primer for ID2839 cloning
aggagatataccatggcggcgtacaccaagccgtc

SEQ ID NO: 25 - DNA, 35 bp, Artificial Sequence
  R primer for ID2839 cloning
gtggtggtgctcgagttagtaggtgaattgtgcgg

SEQ ID NO: 26 - DNA, 35 bp, Artificial Sequence
  F primer for ID2839 cloning
aggagatataccatggcgtacaccaagccgtccac